European Patent Application EP 4 512 891 A1, published February 26, 2025. Title: Transaminase Mutant and Use Thereof. Applicant: ASYMCHEM LABORATORIES(TIANJIN) CO.,LTD. The sequence listing filed with the application follows.

SEQUENCE LISTING (2 sequences)

SEQ ID NO: 1 - protein, 350 aa, Sciscionella sp.
MTTTEFANREIHMTTTEFANSNLVAVEPVAIREPTPPGSVIQYSEYELDRSHPLAGGVAWIEGEYVPADEARISIFDMGFYTSDATYTGIHVWHGNIFRLEDHLDRLLHGAARLKLETGMSREELAGIAKRCVSLSQLREAMVNITITRGYGSTPYGRDATKHRPQVYVYAIPYQWIFPPEEQIFGTSVIVPRHVRRAGLNTIDPTIKNFQWGDLSAAIREAHDRGARSAVLLDADNCVAEGPGFNVVLVKDGALVSPSRNALPGITRKTVYEIAAAKGIETMLRDVTSSELYEADELMAVSTGGGVTPITSLDGEQVGNGEPGPITVAIRDRFWALMDEPSSLIEAIDY

SEQ ID NO: 2 - DNA, 1053 bp, Sciscionella sp.
atgaccaccaccgagtttgccaacagggaattccatatgaccaccaccgagtttgccaacagcaatctggtggccgtggaaccggttgcaatccgtgagcctacccctccgggcagcgtgattcagtacagcgagtacgaactggatcgcagccatccgctggcaggtggcgttgcctggattgaaggcgagtatgttcctgccgatgaagcccgtatcagcatcttcgatatgggcttttataccagcgatgcgacctataccgggatccacgtttggcacggcaatatcttccgcctggaagaccacctggaccgcctgctgcatggtgccgcacgtctgaaactggaaaccggtatgagccgcgaagaactggccggcattgccaagcgttgtgttagcctgagccagctgcgcgaagccatggtgaacatcaccattacccgcggctatggcagcaccccctacggaagggatgcgaccaaacataggccccaggtgtacgtgtatgccatcccgtatcagtggatcttccctccggaggaacagattttcggcaccagcgtgattgtgccgcgtcatgtgcgccgcgccggtctcaataccatcgacccgaccatcaagaactttcagtggggtgacctgtccgccgccatccgtgaggcccatgatcgcggcgcacgtagcgcagttctgctggatgccgataattgcgtggccgagggtccgggctttaatgtggttctggtgaaggacggcgcactggtgagtccgagtcgtaacgcactgccgggcatcacccgcaaaaccgtgtacgaaatcgcagcagccaaaggcatcgaaaccatgctgcgcgacgtgaccagcagtgaactgtatgaggcagatgagctgatggccgtgagcaccggaggtggtgtgacccctattaccagcctggatggcgagcaggttggcaacggtgagccgggcccgattaccgtggccattcgtgatcgcttttgggcactgatggatgagccgagcagcctgattgaggccattgactattaa